European Patent Specification EP 4 049 673 B1, published January 28, 2026. Title: COMPOSITIONS AND MEDICAL USES THEREOF. Applicant: THE TRUSTEES OF THE UNIVERSITY OF PENNSYLVANIA CHILDREN'S HOSPITAL OF PHILADELPHIA. The sequence listing filed with the application follows.

SEQUENCE LISTING (10 sequences)

SEQ ID NO: 1 - protein, 31 aa, Heloderma suspectum
  MOD-RES (31)..(31): AMIDATION
DLSKQMEEEAVRLFIEWLKNGGPSSGAPPPS

SEQ ID NO: 2 - protein, 87 aa, Heloderma suspectum
MKIILWLCVFGLFLATLFPVSWQMPVESGLSSEDSASSESFASKIKRHSDGTFTSDLSKQMEEEAVRLFIEWLKNGGPSSGAPPPSG

SEQ ID NO: 3 - protein, 40 aa, Heloderma suspectum
GEGTFTSQLSKQMEEEAVRLFIEWLKNGGPSSGAPPPSNH

SEQ ID NO: 4 - protein, 41 aa, Heloderma suspectum
KRHSDGTFTSDLSKQMEEEAVRLFIEWLKNGGPSSGAPPPS

SEQ ID NO: 5 - protein, 30 aa, Heloderma suspectum
HAEGTFTSDVSSYLEGQAAKEFIAWLVKGR

SEQ ID NO: 6 - protein, 30 aa, Heloderma suspectum
HAEGTFTSKVSSYLEGQAAKEFIAWLVKGR

SEQ ID NO: 7 - protein, 41 aa, Heloderma suspectum
HGEGTFTSDLSKQMEEEAVRLFIEWLKNGGPSSGAPPPSNH

SEQ ID NO: 8 - protein, 40 aa, Heloderma suspectum
GEGTFTSELSKQMEEEAVRLFIEWLKNGGPSSGAPPPSNH

SEQ ID NO: 9 - protein, 30 aa, Heloderma suspectum; identical to SEQ ID NO: 5

SEQ ID NO: 10 - protein, 39 aa, Heloderma suspectum
  MOD_RES (39)..(39): AMIDATION
HSDGTFTSDLSKGMEEEAVRLFIEWLKNGGPSSGAPPPS